European Patent Specification EP 3 494 236 B1, published March 1, 2023. Title: METHOD FOR CONDUCTING EARLY DETECTION OF COLON CANCER AND/OR OF COLON CANCER PRECURSOR CELLS AND FOR MONITORING COLON CANCER RECURRENCE. Applicant: DIACARTA LLC. The sequence listing filed with the application follows.

SEQUENCE LISTING (56 sequences)

SEQ ID NO: 1 - DNA, 95 bp, Artificial
  Synthetic
  modified_base (1)..(95): Biotinylated capture probe
gatacagctaattcagaatcattttgtggacgaatatgatccaacaatagaggtaaatcttgttttaatatgcatattactggtgcaggaccatt

SEQ ID NO: 2 - DNA, 90 bp, Artificial
  Synthetic
  modified_base (1)..(90): Biotinylated capture probe
aagtcaatcatccacagagacctcaagagtaataatatatttcttcatgaagacctcacagtaaaaataggtgattttggtctagctaca

SEQ ID NO: 3 - DNA, 63 bp, Artificial
  Synthetic
  modified_base (1)..(63): Biotinylated capture probe
aggaaggaaggctggaagagtgcctcagggcagcggaaccgctcattgccaatggtgatgacc

SEQ ID NO: 4 - DNA, 80 bp, Artificial
  Synthetic
  modified_base (1)..(80): Biotinylated capture probe
ttgtcatcagctgaagatgaaataggatgtaatcagacgacacaggaagcagattctgctaataccctgcaaatagcaga

SEQ ID NO: 5 - DNA, 75 bp, Artificial
  Synthetic
  modified_base (1)..(75): Biotinylated capture probe
gtaaaggcaatcctgaggaagaggatgtggatacctcccaagtcctgtatgagtgggaacagggattttctcagt

SEQ ID NO: 6 - DNA, 19 bp, Artificial
  Synthetic
gaatcagctccatccaagt

SEQ ID NO: 7 - DNA, 23 bp, Artificial
  Synthetic
ctgtgacactgctggaacttcgc

SEQ ID NO: 8 - DNA, 25 bp, Artificial
  Synthetic
agcaccctagaaccaaatccagcag

SEQ ID NO: 9 - DNA, 20 bp, Artificial
  Synthetic
tggcatggtttgtccagggc

SEQ ID NO: 10 - DNA, 22 bp, Artificial
  Synthetic
acaaaccatgccaccaagcaga

SEQ ID NO: 11 - DNA, 24 bp, Artificial
  Synthetic
gagcactcaggctggatgaacaag

SEQ ID NO: 12 - DNA, 23 bp, Artificial
  Synthetic
ggatgtaatcagacgacacagga

SEQ ID NO: 13 - DNA, 25 bp, Artificial
  Synthetic
cacaggatcttcatctgacctagtt

SEQ ID NO: 14 - DNA, 19 bp, Artificial
  Synthetic
tctccctccaaaagtggtg

SEQ ID NO: 15 - DNA, 25 bp, Artificial
  Synthetic
aaactatcaagtgaactgacagaag

SEQ ID NO: 16 - DNA, 21 bp, Artificial
  Synthetic
ccagatagccctggacaaacc

SEQ ID NO: 17 - DNA, 28 bp, Artificial
  Synthetic
cttttcagcagtaggtgctttattttta

SEQ ID NO: 18 - DNA, 22 bp, Artificial
  Synthetic
actctggaatccattctggtgc

SEQ ID NO: 19 - DNA, 24 bp, Artificial
  Synthetic
agaaaatccctgttcccactcata

SEQ ID NO: 20 - DNA, 20 bp, Artificial
  Synthetic
atccattctggtgccactac

SEQ ID NO: 21 - DNA, 20 bp, Artificial
  Synthetic
acttgggaggtatccacatc

SEQ ID NO: 22 - DNA, 21 bp, Artificial
  Synthetic
acgacacaggaagcagattct

SEQ ID NO: 23 - DNA, 22 bp, Artificial
  Synthetic
tcacaggatcttcagctgacct

SEQ ID NO: 24 - DNA, 24 bp, Artificial
  Synthetic
ttccaatcttttatttctgctatt

SEQ ID NO: 25 - DNA, 24 bp, Artificial
  Synthetic
  modified_base (1)..(24): Lys modified base
ctgacctagttccaatcttttctt

SEQ ID NO: 26 - DNA, 19 bp, Artificial
  Synthetic
ttcaggagcgaaatctccc

SEQ ID NO: 27 - DNA, 19 bp, Artificial
  Synthetic
tgaacatagtgttcaggtg

SEQ ID NO: 28 - DNA, 28 bp, Artificial
  Synthetic
  modified_base (1)..(28): Fluorescent modified probe
caaaagtggtgcttagacacccaaaagt

SEQ ID NO: 29 - DNA, 15 bp, Artificial
  Synthetic
  modified_base (1)..(15): Lys modified base
agtggtgctcagaca

SEQ ID NO: 30 - DNA, 21 bp, Artificial
  Synthetic
ccagatagccctggacaaacc

SEQ ID NO: 31 - DNA, 28 bp, Artificial
  Synthetic
cttttcagcagtaggtgctttattttta

SEQ ID NO: 32 - DNA, 20 bp, Artificial
  Synthetic
aggtacttctcacttggttt

SEQ ID NO: 33 - DNA, 21 bp, Artificial
  Synthetic
taggtacttctcgcttggttt

SEQ ID NO: 34 - DNA, 22 bp, Artificial
  Synthetic
actctggaatccattctggtgc

SEQ ID NO: 35 - DNA, 24 bp, Artificial
  Synthetic
agaaaatccctgttcccactcata

SEQ ID NO: 36 - DNA, 27 bp, Artificial
  Synthetic
aggaagaggatgtggatacctcccaag

SEQ ID NO: 37 - DNA, 17 bp, Artificial
  Synthetic
  modified_base (1)..(17): Lys modified base
tgccactaccacagctc

SEQ ID NO: 38 - DNA, 22 bp, Artificial
  Synthetic
actctggaatccattctggtgc

SEQ ID NO: 39 - DNA, 24 bp, Artificial
  Synthetic
agaaaatccctgttcccactcata

SEQ ID NO: 40 - DNA, 27 bp, Artificial
  Synthetic
aggaagaggatgtggatacctcccaag

SEQ ID NO: 41 - DNA, 15 bp, Artificial
  Synthetic
  modified_base (1)..(15): Acetyl modified base
ctccttctctgagtg

SEQ ID NO: 42 - DNA, 21 bp, Artificial
  Synthetic
aaggcctgctgaaaatgactg

SEQ ID NO: 43 - DNA, 20 bp, Artificial
  Synthetic
gttggatcatattcgtccac

SEQ ID NO: 44 - DNA, 29 bp, Artificial
  Synthetic
tctgaattagctgtatcgtcaaggcactc

SEQ ID NO: 45 - DNA, 24 bp, Artificial
  Synthetic
  modified_base (1)..(24): D-Lys modified base
ctacgccaccagctccaactacca

SEQ ID NO: 46 - DNA, 22 bp, Artificial
  Synthetic
acttgtggtagttggagctggt

SEQ ID NO: 47 - DNA, 20 bp, Artificial
  Synthetic
gttggatcatattcgtccac

SEQ ID NO: 48 - DNA, 29 bp, Artificial
  Synthetic
tctgaattagctgtatcgtcaaggcactc

SEQ ID NO: 49 - DNA, 23 bp, Artificial
  Synthetic
  modified_base (1)..(23): D-Lys PEG modified base
tcttgcctacgccaccagctcca

SEQ ID NO: 50 - DNA, 31 bp, Artificial
  Synthetic
acagtaaaaataggtgattttggtctagcta

SEQ ID NO: 51 - DNA, 24 bp, Artificial
  Synthetic
catccacaaaatggatccagacaa

SEQ ID NO: 52 - DNA, 25 bp, Artificial
  Synthetic
caaactgatgggacccactccatcg

SEQ ID NO: 53 - DNA, 24 bp, Artificial
  Synthetic
atcgagatttcactgtagctagac

SEQ ID NO: 54 - DNA, 20 bp, Artificial
  Synthetic
cctggacttcgagcaagaga

SEQ ID NO: 55 - DNA, 17 bp, Artificial
  Synthetic
ccgtcaggcagctcgta

SEQ ID NO: 56 - DNA, 22 bp, Artificial
  Synthetic
cttccagctcctccctggagaa